European Patent Application EP 4 741 499 A1, published May 13, 2026. Title: PROTECTED DNA AND METHODS FOR THE PRODUCTION THEREOF. Applicant: 4basebio UK Ltd. Application EP. The sequence listing filed with the application follows.

SEQUENCE LISTING (31 sequences)

SEQ ID NO: 1 - DNA, 16 bp, synthetic construct
  source 1..16: mol_type = other DNA
  modified_base 1..5: mod_base = OTHER; note = nuclease resistant nucleotide
ggccaacaaatgttag

SEQ ID NO: 2 - DNA, 20 bp, synthetic construct
  source 1..20: mol_type = other DNA
nnnnctaacatttgttggcc

SEQ ID NO: 3 - DNA, 20 bp, synthetic construct
  source 1..20: mol_type = other DNA
  modified_base 16..20: mod_base = OTHER; note = nuclease resistant nucleotide
nnnnctaacatttgttggcc

SEQ ID NO: 4 - DNA, 16 bp, synthetic construct
  source 1..16: mol_type = other DNA
ggccaacaaatgttag

SEQ ID NO: 5 - DNA, 21 bp, synthetic construct
  source 1..21: mol_type = other DNA
  modified_base 1..5: mod_base = OTHER; note = nuclease resistant nucleotide
ggccaacaaatgttagnnnnn

SEQ ID NO: 6 - DNA, 21 bp, synthetic construct
  source 1..21: mol_type = other DNA
nnnnnctaacatttgttggcc

SEQ ID NO: 7 - DNA, 12 bp, synthetic construct
  source 1..12: mol_type = other DNA
  modified_base 1: mod_base = OTHER; note = nuclease resistant nucleotide
nacaaatgttag

SEQ ID NO: 8 - DNA, 16 bp, synthetic construct
  source 1..16: mol_type = other DNA
agggctaacatttgtn

SEQ ID NO: 9 - DNA, 16 bp, synthetic construct
  source 1..16: mol_type = other DNA
  modified_base 16: mod_base = OTHER; note = nuclease resistant nucleotide
agggctaacatttgtn

SEQ ID NO: 10 - DNA, 15 bp, synthetic construct
  source 1..15: mol_type = other DNA
  modified_base 15: mod_base = OTHER; note = nuclease resistant nucleotide
catgctaacatttgn

SEQ ID NO: 11 - DNA, 11 bp, synthetic construct
  source 1..11: mol_type = other DNA
ncaaatgttag

SEQ ID NO: 12 - DNA, 11 bp, synthetic construct
  source 1..11: mol_type = other DNA
  modified_base 1: mod_base = OTHER; note = nuclease resistant nucleotide
ncaaatgttag

SEQ ID NO: 13 - DNA, 34 bp, synthetic construct
  source 1..34: mol_type = other DNA
ataacttcgtatagcatacattatacgaagttat

SEQ ID NO: 14 - DNA, 21 bp, synthetic construct
  source 1..21: mol_type = other DNA
  modified_base 17..21: mod_base = OTHER; note = nuclease resistant nucleotide
nnnnnctaacatttgttggcc

SEQ ID NO: 15 - DNA, 21 bp, synthetic construct
  source 1..21: mol_type = other DNA
ggccaacaaatgttagnnnnn

SEQ ID NO: 16 - DNA, 16 bp, synthetic construct
  source 1..16: mol_type = other DNA
  modified_base 1..5: mod_base = OTHER; note = nuclease resistant nucleotide
cgcgcagtgacacccc

SEQ ID NO: 17 - DNA, 20 bp, synthetic construct
  source 1..20: mol_type = other DNA
atctggggtgtcactgcgcg

SEQ ID NO: 18 - DNA, 18 bp, synthetic construct
  source 1..18: mol_type = other DNA
  modified_base 14..18: mod_base = OTHER; note = nuclease resistant nucleotide
gggagggtcgggacaaag

SEQ ID NO: 19 - DNA, 14 bp, synthetic construct
  source 1..14: mol_type = other DNA
ctttgtcccgaccc

SEQ ID NO: 20 - DNA, 16 bp, synthetic construct
  source 1..16: mol_type = other DNA
  modified_base 1..5: mod_base = OTHER; note = nuclease resistant nucleotide
ggccaagaaaagttag

SEQ ID NO: 21 - DNA, 19 bp, synthetic construct
  source 1..19: mol_type = other DNA
  modified_base 9..11: mod_base = OTHER; note = uracil
  modified_base 15..19: mod_base = OTHER; note = nuclease resistant nucleotide
agggctaatttacttggcc

SEQ ID NO: 22 - DNA, 16 bp, synthetic construct
  source 1..16: mol_type = other DNA
  modified_base 1..5: mod_base = OTHER; note = nuclease resistant nucleotide
ggccaagtaaagttag

SEQ ID NO: 23 - DNA, 20 bp, synthetic construct
  source 1..20: mol_type = other DNA
agggctaactttacttggcc

SEQ ID NO: 24 - DNA, 16 bp, synthetic construct
  source 1..16: mol_type = other DNA
  modified_base 1..5: mod_base = OTHER; note = nuclease resistant nucleotide
ggccaagtaaagttag

SEQ ID NO: 25 - DNA, 20 bp, synthetic construct
  source 1..20: mol_type = other DNA
  modified_base 9: mod_base = OTHER; note = uracil
  modified_base 14: mod_base = OTHER; note = uracil
agggctattgttttgtggcc

SEQ ID NO: 26 - DNA, 16 bp, synthetic construct
  source 1..16: mol_type = other DNA
  modified_base 1..5: mod_base = OTHER; note = nuclease resistant nucleotide
ggccaaataaaattag

SEQ ID NO: 27 - DNA, 20 bp, synthetic construct
  source 1..20: mol_type = other DNA
  modified_base 9: mod_base = OTHER; note = uracil
  modified_base 14: mod_base = OTHER; note = uracil
agggctaattttatttggcc

SEQ ID NO: 28 - DNA, 20 bp, synthetic construct
  source 1..20: mol_type = other DNA
  modified_base 16..20: mod_base = OTHER; note = nuclease resistant nucleotide
ttttctaacatttgttggcc

SEQ ID NO: 29 - DNA, 16 bp, synthetic construct
  source 1..16: mol_type = other DNA
  modified_base 1..5: mod_base = OTHER; note = nuclease resistant nucleotide
ggccaacaaatgttag

SEQ ID NO: 30 - DNA, 20 bp, synthetic construct
  source 1..20: mol_type = other DNA
  modified_base 16..20: mod_base = OTHER; note = nuclease resistant nucleotide
ttttctaacatttgttggcc

SEQ ID NO: 31 - DNA, 16 bp, synthetic construct
  source 1..16: mol_type = other DNA
ggccaacaaatgttag